European Patent Specification EP 3 643 333 B1, published May 10, 2023. Title: An assembled biomaterial for bone tissue regeneration and method for preparing the same. Applicant: NANO INTELLIGENT BIOMEDICAL ENGINEERING CORPORATION. CO. LTD SEOUL NATIONAL UNIVERSITY R&DB FOUNDATION. The sequence listing filed with the application follows.

SEQUENCE LISTING (3 sequences)

SEQ ID NO: 1 - protein, 15 aa, Artificial Sequence
  human beta-defensin derived peptide(BD3-3)
GKCSTRGRKCCRRKK

SEQ ID NO: 2 - protein, 15 aa, Artificial Sequence
  human beta-defensin derived peptide(BD3-3-M1)
GKCSTRGRKCMRRKK

SEQ ID NO: 3 - protein, 15 aa, Artificial Sequence
  human beta-defensin derived peptide(BD3-3-M2)
GKCSTRGRKMCRRKK